European Patent Application EP 4 311 558 A2, published January 31, 2024. Title: ANTIBODIES THAT BIND IL-23. Applicant: Eli Lilly and Company. Application EP. The sequence listing filed with the application follows.

SEQUENCE LISTING (15 sequences)

SEQ ID NO: 1 - protein, 10 aa, synthetic construct
  REGION 1..10: note = synthetic construct
GYKFTRYVMH

SEQ ID NO: 2 - protein, 17 aa, synthetic construct
  REGION 1..17: note = synthetic construct
YINPYNDGTNYNEKFKG

SEQ ID NO: 3 - protein, 8 aa, synthetic construct
  REGION 1..8: note = synthetic construct
ARNWDTGL

SEQ ID NO: 4 - protein, 11 aa, synthetic construct
  REGION 1..11: note = synthetic construct
KASDHILKFLT

SEQ ID NO: 5 - protein, 7 aa, synthetic construct
  REGION 1..7: note = synthetic construct
GATSLET

SEQ ID NO: 6 - protein, 9 aa, synthetic construct
  REGION 1..9: note = synthetic construct
QMYWSTPFT

SEQ ID NO: 7 - protein, 115 aa, synthetic construct
  REGION 1..115: note = synthetic construct
QVQLVQSGAEVKKPGSSVKVSCKASGYKFTRYVMHWVRQAPGQGLEWMGYINPYNDGTNYNEKFKGRVTITADKSTSTAYMELSSLRSEDTAVYYCARNWDTGLWGQGTTVTVSS

SEQ ID NO: 8 - protein, 107 aa, synthetic construct
  REGION 1..107: note = synthetic construct
DIQMTQSPSSLSASVGDRVTITCKASDHILKFLTWYQQKPGKAPKLLIYGATSLETGVPSRFSGSGSGTDFTLTISSLQPEDFATYYCQMYWSTPFTFGGGTKVEIK

SEQ ID NO: 9 - protein, 441 aa, synthetic construct
  REGION 1..441: note = synthetic construct
QVQLVQSGAEVKKPGSSVKVSCKASGYKFTRYVMHWVRQAPGQGLEWMGYINPYNDGTNYNEKFKGRVTITADKSTSTAYMELSSLRSEDTAVYYCARNWDTGLWGQGTTVTVSSASTKGPSVFPLAPCSRSTSESTAALGCLVKDYFPEPVTVSWNSGALTSGVHTFPAVLQSSGLYSLSSVVTVPSSSLGTKTYTCNVDHKPSNTKVDKRVESKYGPPCPPCPAPEAAGGPSVFLFPPKPKDTLMISRTPEVTCVVVDVSQEDPEVQFNWYVDGVEVHNAKTKPREEQFNSTYRVVSVLTVLHQDWLNGKEYKCKVSNKGLPSSIEKTISKAKGQPREPQVYTLPPSQEEMTKNQVSLTCLVKGFYPSDIAVEWESNGQPENNYKTTPPVLDSDGSFFLYSRLTVDKSRWQEGNVFSCSVMHEALHNHYTQKSLSLSLG

SEQ ID NO: 10 - protein, 214 aa, synthetic construct
  REGION 1..214: note = synthetic construct
DIQMTQSPSSLSASVGDRVTITCKASDHILKFLTWYQQKPGKAPKLLIYGATSLETGVPSRFSGSGSGTDFTLTISSLQPEDFATYYCQMYWSTPFTFGGGTKVEIKRTVAAPSVFIFPPSDEQLKSGTASVVCLLNNFYPREAKVQWKVDNALQSGNSQESVTEQDSKDSTYSLSSTLTLSKADYEKHKVYACEVTHQGLSSPVTKSFNRGEC

SEQ ID NO: 11 - DNA, 345 bp, synthetic construct
  misc_feature 1..345: note = synthetic construct
  source 1..345: mol_type = other DNA
caggtgcagctggtgcagtctggggctgaggtgaagaagcctgggtcctcggtgaaggtctcctgcaaggcttctggatataaattcactcgttatgttatgcactgggtgcgacaggcccctggacaagggcttgagtggatgggatatattaatccttacaatgatggtactaactacaatgagaagttcaaaggcagagtcacgattaccgcggacaaatccacgagcacagcctacatggagctgagcagcctgagatctgaggacacggccgtgtattactgtgcgagaaactgggacacaggcctctggggccaaggcaccactgtcacagtctcctca

SEQ ID NO: 12 - DNA, 321 bp, synthetic construct
  misc_feature 1..321: note = synthetic construct
  source 1..321: mol_type = other DNA
gacatccagatgacccagtctccatcctccctgtctgcatctgtaggagacagagtcaccatcacttgcaaggcaagtgaccacattctcaaatttttaacttggtatcagcagaaaccagggaaagcccctaagctcctgatctatggtgcaaccagtttggaaactggggtcccatcaaggttcagtggcagtggatctgggacagatttcactctcaccatcagcagtctgcaacctgaagattttgcaacttactactgtcaaatgtattggagtactccgttcacgttcggaggggggaccaaggtggaaataaaa

SEQ ID NO: 13 - DNA, 1323 bp, synthetic construct
  misc_feature 1..1323: note = synthetic construct
  source 1..1323: mol_type = other DNA
caggtgcagctggtgcagtctggggctgaggtgaagaagcctgggtcctcggtgaaggtctcctgcaaggcttctggatataaattcactcgttatgttatgcactgggtgcgacaggcccctggacaagggcttgagtggatgggatatattaatccttacaatgatggtactaactacaatgagaagttcaaaggcagagtcacgattaccgcggacaaatccacgagcacagcctacatggagctgagcagcctgagatctgaggacacggccgtgtattactgtgcgagaaactgggacacaggcctctggggccaaggcaccactgtcacagtctcctcagcctccaccaagggcccatcggtcttcccgctagcgccctgctccaggagcacctccgagagcacagccgccctgggctgcctggtcaaggactacttccccgaaccggtgacggtgtcgtggaactcaggcgccctgaccagcggcgtgcacaccttcccggctgtcctacagtcctcaggactctactccctcagcagcgtggtgaccgtgccctccagcagcttgggcacgaagacctacacctgcaacgtagatcacaagcccagcaacaccaaggtggacaagagagttgagtccaaatatggtcccccatgcccaccctgcccagcacctgaggccgccgggggaccatcagtcttcctgttccccccaaaacccaaggacactctcatgatctcccggacccctgaggtcacgtgcgtggtggtggacgtgagccaggaagaccccgaggtccagttcaactggtacgtggatggcgtggaggtgcataatgccaagacaaagccgcgggaggagcagttcaacagcacgtaccgtgtggtcagcgtcctcaccgtcctgcaccaggactggctgaacggcaaggagtacaagtgcaaggtctccaacaaaggcctcccgtcctccatcgagaaaaccatctccaaagccaaagggcagccccgagagccacaggtgtacaccctgcccccatcccaggaggagatgaccaagaaccaggtcagcctgacctgcctggtcaaaggcttctaccccagcgacatcgccgtggagtgggaaagcaatgggcagccggagaacaactacaagaccacgcctcccgtgctggactccgacggctccttcttcctctacagcaggctaaccgtggacaagagcaggtggcaggaggggaatgtcttctcatgctccgtgatgcatgaggctctgcacaaccactacacacagaagagcctctccctgtctctgggt

SEQ ID NO: 14 - DNA, 642 bp, synthetic construct
  misc_feature 1..642: note = synthetic construct
  source 1..642: mol_type = other DNA
gacatccagatgacccagtctccatcctccctgtctgcatctgtaggagacagagtcaccatcacttgcaaggcaagtgaccacattctcaaatttttaacttggtatcagcagaaaccagggaaagcccctaagctcctgatctatggtgcaaccagtttggaaactggggtcccatcaaggttcagtggcagtggatctgggacagatttcactctcaccatcagcagtctgcaacctgaagattttgcaacttactactgtcaaatgtattggagtactccgttcacgttcggaggggggaccaaggtggaaataaaacgaactgtggctgcaccatctgtcttcatcttcccgccatctgatgagcagttgaaatctggaactgcctctgttgtgtgcctgctgaataacttctatcccagagaggccaaagtacagtggaaggtggataacgccctccaatcgggtaactcccaggagagtgtcacagagcaggacagcaaggacagcacctacagcctcagcagcaccctgacgctgagcaaagcagactacgagaaacacaaagtctacgcctgcgaagtcacccatcagggcctgagctcgcccgtcacaaagagcttcaacaggggagagtgc

SEQ ID NO: 15 - protein, 170 aa, Homo sapiens
RAVPGGSSPAWTQCQQLSQKLCTLAWSAHPLVGHMDLREEGDEETTNDVPHIQCGDGCDPQGLRDNSQFCLQRIHQGLIFYEKLLGSDIFTGEPSLLPDSPVGQLHASLLGLSQLLQPEGHHWETQQIPSLSPSQPWQRLLLRFKILRSLQAFVAVAARVFAHGAATLSP